European Patent Application EP 4 600 411 A2, published August 13, 2025. Title: VERSATILE PEPTIDE AND PROTEIN MACROCYCLIZATION AND MULTIMERIZATION WITH DIELS-ALDER CYCLOADDITIONS. Applicant: The University of Chicago. Application EP. The sequence listing filed with the application follows.

SEQUENCE LISTING (37 sequences)

SEQ ID NO: 1-2 - skipped (2 entries)

SEQ ID NO: 3 - protein, 6 aa, synthetic construct
  REGION 1..6: note = synthetic
  SITE 1: note = MISC_FEATURE - Xaa is C(hex)
  SITE 6: note = MISC_FEATURE - Xaa is K(mal)
XAPVYX

SEQ ID NO: 4 - protein, 8 aa, synthetic construct
  REGION 1..8: note = synthetic
  SITE 1: note = MISC_FEATURE - Xaa is C(hex)
  SITE 8: note = MISC_FEATURE - Xaa is K(mal)
XAVPAVYX

SEQ ID NO: 5 - skipped

SEQ ID NO: 6 - protein, 21 aa, synthetic construct
  REGION 1..21: note = synthetic
SCFGGRMDRIGAQSGLGCNSF

SEQ ID NO: 7 - protein, 21 aa, synthetic construct
  REGION 1..21: note = synthetic
  SITE 7: note = MISC_FEATURE - Xaa is AA with dienophile
  SITE 14: note = MISC_FEATURE - Xaa is AA with diene
SCFGGRXDRIGAQXGLGCNSF

SEQ ID NO: 8 - protein, 21 aa, synthetic construct
  REGION 1..21: note = synthetic
  SITE 7: note = MISC_FEATURE - Xaa is C(hex)
  SITE 14: note = MISC_FEATURE - Xaa is K(mal)
SCFGGRXDRIGAQXGLGCNSF

SEQ ID NO: 9 - protein, 24 aa, synthetic construct
  REGION 1..24: note = synthetic
  SITE 22: note = MISC_FEATURE - Xaa is beta-alanine
  SITE 23: note = MISC_FEATURE - Xaa is K(mmt)
KRAHHNALERKRRDHIKDSFHXXW

SEQ ID NO: 10 - protein, 21 aa, synthetic construct
  REGION 1..21: note = synthetic
  SITE 3: note = MISC_FEATURE - Xaa is S5
  SITE 7: note = MISC_FEATURE - Xaa is S5
  SITE 20: note = MISC_FEATURE - Xaa is beta-alanine
  SITE 21: note = MISC_FEATURE - Xaa is K(mmt)
KRXHHNXLERKRRDHIKDSXX

SEQ ID NO: 11 - protein, 24 aa, synthetic construct
  REGION 1..24: note = synthetic
  SITE 22: note = MISC_FEATURE - Xaa is beta-alanine
  SITE 23: note = MISC_FEATURE - Xaa is K(cpd)
KRAHHNALERKRRDHIKDSFHXXW

SEQ ID NO: 12 - protein, 21 aa, synthetic construct
  REGION 1..21: note = synthetic
  SITE 3: note = MISC_FEATURE - Xaa is S5
  SITE 7: note = MISC_FEATURE - Xaa is S5
  SITE 20: note = MISC_FEATURE - Xaa is beta-alanine
  SITE 21: note = MISC_FEATURE - Xaa is K(cpd)
KRXHHNXLERKRRDHIKDSXX

SEQ ID NO: 13-14 - skipped (2 entries)

SEQ ID NO: 15 - protein, 5 aa, synthetic construct
  REGION 1..5: note = synthetic
CRGDK

SEQ ID NO: 16 - protein, 5 aa, synthetic construct
  REGION 1..5: note = synthetic
  SITE 1: note = MISC_FEATURE - Xaa is C(tBuS)
XVGDK

SEQ ID NO: 17 - protein, 5 aa, synthetic construct
  REGION 1..5: note = synthetic
  SITE 1: note = MISC_FEATURE - Xaa is C(Hex)
XVGDK

SEQ ID NO: 18 - protein, 6 aa, synthetic construct
  REGION 1..6: note = synthetic
  SITE 1: note = MISC_FEATURE - Xaa is C(tBuS)
XAPVYK

SEQ ID NO: 19 - protein, 6 aa, synthetic construct
  REGION 1..6: note = synthetic
  SITE 1: note = MISC_FEATURE - Xaa is C(Hex)
XAPVYK

SEQ ID NO: 20 - protein, 8 aa, synthetic construct
  REGION 1..8: note = synthetic
CAVPAVYK

SEQ ID NO: 21 - protein, 8 aa, synthetic construct
  REGION 1..8: note = synthetic
  SITE 1: note = MISC_FEATURE - Xaa is C(tBuS)
XAVPAVYK

SEQ ID NO: 22 - protein, 8 aa, synthetic construct
  REGION 1..8: note = synthetic
  SITE 1: note = MISC_FEATURE - Xaa is C(Hex)
XAVPAVYK

SEQ ID NO: 23 - protein, 16 aa, synthetic construct
  REGION 1..16: note = synthetic
  SITE 7: note = MISC_FEATURE - Xaa is S5
  SITE 14: note = MISC_FEATURE - Xaa is S5
QSQQTFXNLWRLLXQN

SEQ ID NO: 24 - protein, 16 aa, synthetic construct
  REGION 1..16: note = synthetic
  SITE 14: note = MISC_FEATURE - Xaa is A(Fur)
QSQQTFKNLWRLLXQN

SEQ ID NO: 25 - protein, 16 aa, synthetic construct
  REGION 1..16: note = synthetic
  SITE 7: note = MISC_FEATURE - Xaa is K(mal)
  SITE 14: note = MISC_FEATURE - Xaa is A(Fur)
QSQQTFXNLWRLLXQN

SEQ ID NO: 26 - protein, 11 aa, synthetic construct
  REGION 1..11: note = synthetic
HKILHRLLQDS

SEQ ID NO: 27 - protein, 11 aa, synthetic construct
  REGION 1..11: note = synthetic
  SITE 3: note = MISC_FEATURE - Xaa is K(mal)
  SITE 7: note = MISC_FEATURE - Xaa is A(Fur)
HKXLHRXLQDS

SEQ ID NO: 28 - protein, 11 aa, synthetic construct
  REGION 1..11: note = synthetic
  SITE 3: note = MISC_FEATURE - Xaa is S5
  SITE 6: note = MISC_FEATURE - Xaa is K(mal)
  SITE 7: note = MISC_FEATURE - Xaa is S5
  SITE 10: note = MISC_FEATURE - Xaa is A(Fur)
HKXLHXXLQXS

SEQ ID NO: 29 - protein, 11 aa, synthetic construct
  REGION 1..11: note = synthetic
  SITE 6: note = MISC_FEATURE - Xaa is K(mal)
  SITE 10: note = MISC_FEATURE - Xaa is A(Fur)
HKILHXLLQXS

SEQ ID NO: 30 - protein, 15 aa, synthetic construct
  REGION 1..15: note = synthetic
  SITE 1: note = MISC_FEATURE - Xaa is fitc-b-Ser
XLTERHKILHRLLQE

SEQ ID NO: 31 - protein, 11 aa, synthetic construct
  REGION 1..11: note = synthetic
  SITE 7: note = MISC_FEATURE - Xaa is A(Fur)
HKKLHRXLQDS

SEQ ID NO: 32 - protein, 11 aa, synthetic construct
  REGION 1..11: note = synthetic
  SITE 10: note = MISC_FEATURE - Xaa is A(Fur)
HKILHKLLQXS

SEQ ID NO: 33 - protein, 11 aa, synthetic construct
  REGION 1..11: note = synthetic
  SITE 3: note = MISC_FEATURE - Xaa is S5
  SITE 7: note = MISC_FEATURE - Xaa is S5
  SITE 10: note = MISC_FEATURE - Xaa is A(Fur)
HKXLHKXLQXS

SEQ ID NO: 34 - protein, 19 aa, synthetic construct
  REGION 1..19: note = synthetic
  SITE 1: note = MISC_FEATURE - Xaa is Fmoc-beta-Trp
  SITE 4: note = MISC_FEATURE - Xaa is S5
  SITE 8: note = MISC_FEATURE - Xaa is S5
XPQXILDXHVQEVWRRRRR

SEQ ID NO: 35 - protein, 19 aa, synthetic construct
  REGION 1..19: note = synthetic
  SITE 1: note = MISC_FEATURE - Xaa is beta-Trp
  SITE 4: note = MISC_FEATURE - Xaa is S5
  SITE 8: note = MISC_FEATURE - Xaa is S5
XPQXILDXHVQEVWRRRRR

SEQ ID NO: 36 - protein, 196 aa, synthetic construct
  REGION 1..196: note = synthetic
HHHHHHSSGLVPRGSHMGNGTEEDYNFVFKVVLIGESGVGKTNLLSRFTRNEFSHDSRTTIGVEFSTRTVMLGTAAVKAQIWDTAGLERYRAITSAYYRGAVGALLVFDLTKHQTYAVVERWLKELYDHAEATIVVMLVGNKSDLSQAREVPTEEARMFAENNGLLFLETSALDSTNVELAFETVLKEIFAKVSKQ

SEQ ID NO: 37 - protein, 196 aa, synthetic construct
  REGION 1..196: note = synthetic
  SITE 26: note = misc_feature - Xaa is TAG site
  SITE 194: note = misc_feature - Xaa is TAG site
HHHHHHSSGLVPRGSHMGNGTEEDYXFVFKVVLIGESGVGKTNLLSRFTRNEFSHDSRTTIGVEFSTRTVMLGTAAVKAQIWDTAGLERYRAITSAYYRGAVGALLVFDLTKHQTYAVVERWLKELYDHAEATIVVMLVGNKSDLSQAREVPTEEARMFAENNGLLFLETSALDSTNVELAFETVLKEIFAKVXKQ